European Patent Application EP 4 169 939 A2, published April 26, 2023. Title: ANTICORPO, SEU USO, COMPOSIÇÃO FARMACÊUTICA O COMPREENDENDO, MÉTODO DE DIAGNÓSTICO DE INFECÇÕES FÚNGICAS, KIT DE DIAGNÓSTICO DE INFECÇÕES FÚNGICAS E MÉTODO PARA TRATAMENTO DE INFECÇÕES FÚNGICAS. Applicant: Fundação Oswaldo Cruz. The sequence listing filed with the application follows.

SEQUENCE LISTING (20 sequences)

SEQ ID NO: 1 - protein, 10 aa, Mus musculus
GFTFSDYGMA

SEQ ID NO: 2 - protein, 9 aa, Mus musculus
ISNLAYSIY

SEQ ID NO: 3 - protein, 12 aa, Mus musculus
DYYGSSYWYFDV

SEQ ID NO: 4 - protein, 10 aa, Mus musculus
SASSSVSYMH

SEQ ID NO: 5 - protein, 7 aa, Mus musculus
STSNLAS

SEQ ID NO: 6 - protein, 9 aa, Mus musculus
QQRSSYPLT

SEQ ID NO: 7 - protein, 10 aa, Mus musculus
GFTFSDAWMD

SEQ ID NO: 8 - protein, 9 aa, Mus musculus
IRSKANNHA

SEQ ID NO: 9 - protein, 8 aa, Mus musculus
HRYDGFDY

SEQ ID NO: 10 - protein, 10 aa, Mus musculus
SASSSISYMH

SEQ ID NO: 11 - protein, 7 aa, Mus musculus
DTSKLAS

SEQ ID NO: 12 - protein, 8 aa, Mus musculus
QRSSYPCT

SEQ ID NO: 13 - DNA, 373 bp, Mus musculus
ggcagggagcggtgaccgtggtccctgcgccccagacatcgaagtaccagtagctactaccgtagtaatcccttgcacagtagtacatggctgtgtcctcagacctcagactgctcatttccaggtacagggtgttcttggcattctctctagagatggtgaatcggcccgtcacagtgtctgcatagtagatactatatgccaaattactaatgaatgctacccactcaggccccttccctggagcctgtcgaacccacgccattccgtagtcactgaaagtgaatccagaggctgcacaggatagtttccgggaccctccaggctgcactaagcctccccctgactcctccagcttaacttgaccggtcga

SEQ ID NO: 14 - DNA, 331 bp, Mus musculus
gcaaccaattcctgcatctccaggggagaggtcaccataacctgcagtgccagctcaagtgtaagttacatgcactggttccagcagaagccaggcacttctcccaaactctggatttatagcacatccaacctggcttctggagtccctgctcgcttcagtggcagtggatctgggacctcttactctctcacaatcagccgaatggaggctgaagatgctgccacttattactgccagcaaaggagtagttacccgctcacgttcggtgctgggaccaagctggagctgaaacgggctgatgctgcaccaactgtatccctcgagacca

SEQ ID NO: 15 - protein, 124 aa, Mus musculus
STGQVKLEESGGGLVQPGGSRKLSCAASGFTFSDYGMAWVRQAPGKGPEWVAFISNLAYSIYYADTVTGRFTISRENAKNTLYLEMSSLRSEDTAMYYCARDYYGSSYWYFDVWGAGTTVTAPC

SEQ ID NO: 16 - protein, 110 aa, Mus musculus
ATNSCISRGEVTITCSASSSVSYMHWFQQKPGTSPKLWIYSTSNLASGVPARFSGSGSGTSYSLTISRMEAEDAATYYCQQRSSYPLTFGAGTKLELKRADAAPTVSLET

SEQ ID NO: 17 - DNA, 364 bp, Mus musculus
cggggaatgtgagagtggtgccttggccccagtagtcaaagccgtcgtacctatgcctcgtacagtaataaatgccagtgtcttcagctcttaagctgttcatttgcaggtagacactacttttggaatcatctcttgagatggtgaacctccctttcacagactcagcatagtatgttgcatgattattagctttgcttctaatttcagcaacccactcaagccccttctctggagactggcggacccagtccatccaggcgtcactaaaagtgaatccagaggcagcacaagagagtttcatggatcctccaggttgcaccaagcctcctcctgactcctccagcttaacttgaccggtcga

SEQ ID NO: 18 - DNA, 336 bp, Mus musculus
gattattttcttgcatctcagggagaggtcaccatgacctgcagtgccagctcaagtataagttacatgcactggtaccagcagaagccaggcacctcccccaaaagatggatttatgacacatccaaactggcttctggagtccctgctcgcttcagtggcagtgggtctgggacctcttattctctcacaatcagcagcatggaggctgaagatgctgccacttattactgccatcagcggagtagttacccatgcacgttcggtgctgggaccaagctggagctgaaacgggctgatgctgcaccaactgtatccctcgagaccaagaccagc

SEQ ID NO: 19 - protein, 121 aa, Mus musculus
STGQVKLEESGGGLVQPGGSMKLSCAASGFTFSDAWMDWVRQSPEKGLEWVAEIRSKANNHATYYAESVKGRFTISRDDSKSSVYLQMNSLRAEDTGIYYCTRHRYDGFDYWGQGTTLTFP

SEQ ID NO: 20 - protein, 112 aa, Mus musculus
DYFLASQGEVTMTCSASSSISYMHWYQQKPGTSPKRWIYDTSKLASGVPARFSGSGSGTSYSLTISSMEAEDAATYYCHQRSSYPCTFGAGTKLELKRADAAPTVSLETKTS